European Patent Specification EP 3 575 321 B1, published July 26, 2023. Title: CHEMOKINE RECEPTOR BINDING POLYPEPTIDES. Applicant: NOVARTIS AG. The sequence listing filed with the application follows.

SEQUENCE LISTING (248 sequences)

SEQ ID NO: 1 - protein, 360 aa, Homo sapiens
MEDFNMESDSFEDFWKGEDLSNYSYSSTLPPFLLDAAPCEPESLEINKYFVVIIYALVFLLSLLGNSLVMLVILYSRVGRSVTDVYLLNLALADLLFALTLPIWAASKVNGWIFGTFLCKVVSLLKEVNFYSGILLLACISVDRYLAIVHATRTLTQKRYLVKFICLSIWGLSLLLALPVLLFRRTVYSSNVSPACYEDMGNNTANWRMLLRILPQSFGFIVPLLIMLFCYGFTLRTLFKAHMGQKHRAMRVIFAVVLIFLLCWLPYNLVLLADTLMRTQVIQETCERRNHIDRALDATEILGILHSCLNPLIYAFIGQKFRHGLLKILAIHGLISKDSLPKDSRPSFVGSSSGHTSTTL

SEQ ID NO: 2 - protein, 344 aa, Homo sapiens
MEDLSNYSYSSTLPPFLLDAAPCEPESLEINKYFVVIIYALVFLLSLLGNSLVMLVILYSRVGRSVTDVYLLNLALADLLFALTLPIWAASKVNGWIFGTFLCKVVSLLKEVNFYSGILLLACISVDRYLAIVHATRTLTQKRYLVKFICLSIWGLSLLLALPVLLFRRTVYSSNVSPACYEDMGNNTANWRMLLRILPQSFGFIVPLLIMLFCYGFTLRTLFKAHMGQKHRAMRVIFAVVLIFLLCWLPYNLVLLADTLMRTQVIQETCERRNHIDRALDATEILGILHSCLNPLIYAFIGQKFRHGLLKILAIHGLISKDSLPKDSRPSFVGSSSGHTSTTL

SEQ ID NO: 3 - protein, 355 aa, Macaca fascicularis
MQSFNFEDFWENEDFSNYSYSSDLPPSLPDVAPCRPESLEINKYFVVIIYALVFLLSLLGNSLVMLVILHSRVGRSITDVYLLNLAMADLLFALTLPIWAAAKVNGWIFGTFLCKVVSLLKEVNFYSGILLLACISVDRYLAIVHATRTLTQKRYLVKFVCLSIWSLSLLLALPVLLFRRTVYLTYISPVCYEDMGNNTAKWRMVLRILPQTFGFILPLLIMLFCYGFTLRTLFKAHMGQKHRAMRVIFAVVLIFLLCWLPYHLVLLADTLMRTRLINETCQRRNNIDQALDATEILGILHSCLNPLIYAFIGQKFRHGLLKILATHGLISKDSLPKDSRPSFVGSSSGHTSTTL

SEQ ID NO: 4 - protein, 14 aa, Macaca fascicularis
MQSFNFEDFWENED

SEQ ID NO: 5 - protein, 18 aa, Macaca fascicularis
CTLMRTRLINETLQRRNC

SEQ ID NO: 6 - protein, 26 aa, Macaca fascicularis
CRRTVYLTYISPVLYEDMGNNTALWC

SEQ ID NO: 7 - protein, 19 aa, Homo sapiens
MEDFNMESDSFEDFWKGED

SEQ ID NO: 8 - protein, 31 aa, Homo sapiens
EDLSNYSYSSTLPPFLLDAAPCEPESLEINK

SEQ ID NO: 9 - protein, 26 aa, Homo sapiens
FRRTVYSSNVSPACYEDMGNNTANWR

SEQ ID NO: 10 - protein, 26 aa, Homo sapiens
CRRTVYSSNVSPALYEDMGNNTANWC

SEQ ID NO: 11 - protein, 18 aa, Homo sapiens
DTLMRTQVIQETCERRNH

SEQ ID NO: 12 - protein, 18 aa, Homo sapiens
CTLMRTQVIQETLERRNC

SEQ ID NO: 13 - DNA, 21 bp, Artificial Sequence
  PRIMER
ggctgagctgggtggtcctgg

SEQ ID NO: 14 - DNA, 21 bp, Artificial Sequence
  PRIMER
ggctgagtttggtggtcctgg

SEQ ID NO: 15 - DNA, 23 bp, Artificial Sequence
  PRIMER
ggtacgtgctgttgaactgttcc

SEQ ID NO: 16 - DNA, 55 bp, Artificial Sequence
  PRIMER
catttgagttggcctagccggccatggcagaggtgcagctggtggagtctggggg

SEQ ID NO: 17 - DNA, 18 bp, Artificial Sequence
  PRIMER
tgtaaaacgacggccagt

SEQ ID NO: 18 - DNA, 18 bp, Artificial Sequence
  PRIMER
caggaaacagctatgacc

SEQ ID NO: 19 - DNA, 88 bp, Artificial Sequence
  PRIMER
tcagtaacctggatcccccgccaccgctgcctccaccgccgctacccccgccaccgctgcctccaccgcctgaggagacggtgacctg

SEQ ID NO: 20 - DNA, 84 bp, Artificial Sequence
  PRIMER
aggttactgaggatccggcggtggaggcagcggaggtgggggctctggtggcgggggtagcgaggtgcagctggtggagtctgg

SEQ ID NO: 21 - DNA, 24 bp, Artificial Sequence
  PRIMER
gaggtgcaattggtggagtctggg

SEQ ID NO: 22 - DNA, 24 bp, Artificial Sequence
  PRIMER
tgaggagacggtgacctgggtccc

SEQ ID NO: 23 - DNA, 34 bp, Artificial Sequence
  PRIMER
tcttggatccgaggtgcagctggtggagtctggg

SEQ ID NO: 24 - DNA, 33 bp, Artificial Sequence
  PRIMER
accgcctccggaggagaccgtgacctgggtccc

SEQ ID NO: 25 - protein, 119 aa, Artificial Sequence
  monovalent anti-CXCR2 Nanobodies
EVQLVESGGGLVQPGGSLRLSCAASGFTFSTYWMYWVRQAPGKGLDWVSAINAGGDSTYYADPVKGRFTISRDNNKNTLYLQMNSLKPEDTALYYCATVRGTARDLDYWGQGTQVTVSS

SEQ ID NO: 26 - protein, 123 aa, Artificial Sequence
  monovalent anti-CXCR2 Nanobodies
EVKLVESGGGLVQAGGSLRLSCALSGRIGSINAMGWYRQVSGQQRELVAVSRSGGSTDIADSVKGRFTISRDNGKNTVYLQMDSLKPEDTAVYYCYAHTSSYSNWRVYNNDYWGQGTQVTVSS

SEQ ID NO: 27 - protein, 116 aa, Artificial Sequence
  monovalent anti-CXCR2 Nanobodies
EVQLVESGGGLVQAGGSLRLTCAASGRIGTINAMGWYRQAPGKQRELVAVITSGGRIDYADSVKGRFTISRDNAKNTVYLQMNSLKPEDTAVYYYNVETVVGAVYWGQGTQVTVSS

SEQ ID NO: 28 - protein, 116 aa, Artificial Sequence
  monovalent anti-CXCR2 Nanobodies
EVQLVESGGGLVQAGGSLRLSCAASGRMGNINAMGWYRQAPGKERELVAKITRGGAITYADSVKGRFTIARDNILNTAYLQMNDLKPEDTAVYYYNVDGGPSQNYWGQGTQVTVSS

SEQ ID NO: 29 - protein, 126 aa, Artificial Sequence
  monovalent anti-CXCR2 Nanobodies
EVQLVESGGGLVQAGGSLRLSCAASGFTFDDYAIGWFRQAPGKERERVSCISGSDGSTYYADSVKGRFTISSDNAKNTVYLQMNNLKPEDTAVYYCAAYWGLTLRLWMPPHRYDYWGQGTQVTVSS

SEQ ID NO: 30 - protein, 111 aa, Artificial Sequence
  monovalent anti-CXCR2 Nanobodies
EVQLVESGGGLVQAGGSLSLSCAASGLIFRLSGMAWYRQAPGRQREWVAVLTKDGTLHYADPVKGRFTISRNNAENTWYLQMNSLKPEDTAIYYCNTGRYWGQGTQVTVSS

SEQ ID NO: 31 - protein, 115 aa, Artificial Sequence
  monovalent anti-CXCR2 Nanobodies
EVQLVESGGGLVQAGGSLRLSCAASGTIGTIRAMGWYRQAPGKQRELVALITSTGRINYADSVKGRFTIGRDNAKNTAYLQMNNLKPEDTAVYYYNIETLRRNYWGQGTQVTVSS

SEQ ID NO: 32 - protein, 118 aa, Artificial Sequence
  monovalent anti-CXCR2 Nanobodies
EVQLVESGGGLVQAGGSLRLSCAASGRTFSNYAMGWFRQATGKEREFVAAINKSGGNTHYAGSVKGRFTISRDNAKNTVYLQMNSLKPRDTAVYYCAASRTNPKPDYWGQGTQVTVSS

SEQ ID NO: 33 - protein, 122 aa, Artificial Sequence
  monovalent anti-CXCR2 Nanobodies
EVQLVESGGGLVQAGGSLRLSCAASGRSFSRSAMGWLRQAPGKEREFVAGISWGGDNSYYADSVKGRFTISRDNAKNTVSLQMNSLKPQDTAVYYCAARYRGGAAVAGWEYWGQGTQVTVSS

SEQ ID NO: 34 - protein, 124 aa, Artificial Sequence
  monovalent anti-CXCR2 Nanobodies
EVQLVESGGGLVQPGGSLRLSCAASGSTLAYYTVGWFRRAPGKEREGISCISSSDGSTYYADSVKGRFTISRDNAKNTVYLQMNSLKPEDTAVYYCAADRRTDCKKGRVGSGSWGQGTQVTVSS

SEQ ID NO: 35 - protein, 125 aa, Artificial Sequence
  monovalent anti-CXCR2 Nanobodies
KVQLVESGGGLVQAGGSLRLSCAASGRAFNYYVMAWFRQAQGKEREFVAAISTRGSMTKYSDSVQGRFTISRDNAKNTVYLHMNSLKPEDTAVYYCAADPRGSSWSFSSGGYDYWGQGTQVTVSS

SEQ ID NO: 36 - protein, 111 aa, Artificial Sequence
  monovalent anti-CXCR2 Nanobodies
EVQLVESGGGLVQPGGSVRLSCVASGIIFRLSALGWTRQGPGKAREWVAGINSDGTTNYADPVKGRFTISRDNAKNTIYLHMDMLKPEDTAVYYCASGKYRGQGTQVTVSS

SEQ ID NO: 37 - protein, 115 aa, Artificial Sequence
  monovalent anti-CXCR2 Nanobodies
EVQLVESGGGLVQAGESLRLSCAASGSTFDFKVMGWYRQPPGKQREGVAAIRLSGNMHYAESVKGRFTISKANAKNTVYLQMNSLRPEDTAVYYCKVNIRGQDYWGQGTQVTVSS

SEQ ID NO: 38 - protein, 120 aa, Artificial Sequence
  monovalent anti-CXCR2 Nanobodies
EVQLVESGGGLVQAGGSLTLSCAVSGSSFRINTMGWYRRAPGKQRELVAARDRGGYINYVDSVKGRFTVSRDNAKPTMYLQMNSLKPEDTAVYYCHAGTQDRTGRNFDHWGQGTQVTVSS

SEQ ID NO: 39 - protein, 126 aa, Artificial Sequence
  monovalent anti-CXCR2 Nanobodies
EVQLVESGGGLVQPGGSLRLSCVASGSIVRINTMGWYRQTPGKQRELVADITSGGNINYIDAVKGRFTISRDNTKNTVYLQMNSLKPEDTAVYYCNAEIVVLVGVWTQRARTGNYWGQGTQVTVSS

SEQ ID NO: 40 - protein, 124 aa, Artificial Sequence
  monovalent anti-CXCR2 Nanobodies
EVQLVESGGGLVQPGGSLRLSCAASGRTFSSLSMGWFRQAPGKERAFVAALTRNGGYRYYADSVKGRFTISRDVAKKTLYLQMNSLKPEDTAVYYCAADSLSGSDYLGTNLDYWGQGTQVTVSS

SEQ ID NO: 41 - protein, 124 aa, Artificial Sequence
  monovalent anti-CXCR2 Nanobodies
EVQLVESGGGLVQAGGSLRLSCAASGRTFSDYAMGWFRQAPGKEREFVAAITWNGGRVFYTASVKGRFTISRDNAKNTMYLQMNSLKPEDTAVYYCAADKDRRTDYLGHPVAYWGQGTQVTVSS

SEQ ID NO: 42 - protein, 122 aa, Artificial Sequence
  monovalent anti-CXCR2 Nanobodies
EVQLVESGGGLVQPGGSLRLSCVASGRIFSSNAMGWFRQAPGKEREFVAAITWRSGGSAYYADSAKGRFTISRDNAKNTVYLQMNSLKPEDTAVYYCAAGGSSWLSFPPDYWGQGTQVTVSS

SEQ ID NO: 43 - protein, 115 aa, Artificial Sequence
  monovalent anti-CXCR2 Nanobodies
EVQLVESGGELVQPGGSLRLSCAASGSILTINAMGWYRQAPGKQRELVVRRTRGGSTTYQDSVKGRFTISADIAKKTMYLQMNSLKPEDTAVYYCMLDDRGGVYWGQGTQVTVSS

SEQ ID NO: 44 - protein, 287 aa, Artificial Sequence
  multivalent anti-CXCR2 Nanobodies
EVQLVESGGGLVQPGGSLRLSCVASGSIVRINTMGWYRQTPGKQRELVADITSGGNINYIDAVKGRFTISRDNTKNTVYLQMNSLKPEDTAVYYCNAEIVVLVGVWTQRARTGNYWGQGTQVTVSSGGGGSGGGGSGGGGSGGGGSGGGGSGGGGSGGGGSEVQLVESGGGLVQPGGSLRLSCVASGSIVRINTMGWYRQTPGKQRELVADITSGGNINYIDAVKGRFTISRDNTKNTVYLQMNSLKPEDTAVYYCNAEIVVLVGVWTQRARTGNYWGQGTQVTVSS

SEQ ID NO: 45 - protein, 257 aa, Artificial Sequence
  multivalent anti-CXCR2 Nanobodies
EVQLVESGGGLVQPGGSVRLSCVASGIIFRLSALGWTRQGPGKAREWVAGINSDGTTNYADPVKGRFTISRDNAKNTIYLHMDMLKPEDTAVYYCASGKYRGQGTQVTVSSGGGGSGGGGSGGGGSGGGGSGGGGSGGGGSGGGGSEVQLVESGGGLVQPGGSVRLSCVASGIIFRLSALGWTRQGPGKAREWVAGINSDGTTNYADPVKGRFTISRDNAKNTIYLHMDMLKPEDTAVYYCASGKYRGQGTQVTVSS

SEQ ID NO: 46 - protein, 276 aa, Artificial Sequence
  Sequences of multivalent anti-CXCR2 Nanobodies
EVQLVESGGELVQPGGSLRLSCAASGSILTINAMGWYRQAPGKQRELVVRRTRGGSTTYQDSVKGRFTISADIAKKTMYLQMNSLKPEDTAVYYCMLDDRGGVYWGQGTQVTVSSGGGGSGGGGSGGGGSGGGGSGGGGSGGGGSGGGGSEVQLVESGGGLVQPGGSLRLSCVASGSIVRINTMGWYRQTPGKQRELVADITSGGNINYIDAVKGRFTISRDNTKNTVYLQMNSLKPEDTAVYYCNAEIVVLVGVWTQRARTGNYWGQGTQVTVSS

SEQ ID NO: 47 - protein, 276 aa, Artificial Sequence
  Sequences of multivalent anti-CXCR2 Nanobodies
EVQLVESGGGLVQPGGSLRLSCVASGSIVRINTMGWYRQTPGKQRELVADITSGGNINYIDAVKGRFTISRDNTKNTVYLQMNSLKPEDTAVYYCNAEIVVLVGVWTQRARTGNYWGQGTQVTVSSGGGGSGGGGSGGGGSGGGGSGGGGSGGGGSGGGGSEVQLVESGGELVQPGGSLRLSCAASGSILTINAMGWYRQAPGKQRELVVRRTRGGSTTYQDSVKGRFTISADIAKKTMYLQMNSLKPEDTAVYYCMLDDRGGVYWGQGTQVTVSS

SEQ ID NO: 48 - protein, 261 aa, Artificial Sequence
  Sequences of multivalent anti-CXCR2 Nanobodies
EVQLVESGGELVQPGGSLRLSCAASGSILTINAMGWYRQAPGKQRELVVRRTRGGSTTYQDSVKGRFTISADIAKKTMYLQMNSLKPEDTAVYYCMLDDRGGVYWGQGTQVTVSSGGGGSGGGGSGGGGSGGGGSGGGGSGGGGSGGGGSEVQLVESGGGLVQPGGSVRLSCVASGIIFRLSALGWTRQGPGKAREWVAGINSDGTTNYADPVKGRFTISRDNAKNTIYLHMDMLKPEDTAVYYCASGKYRGQGTQVTVSS

SEQ ID NO: 49 - protein, 261 aa, Artificial Sequence
  Sequences of multivalent anti-CXCR2 Nanobodies
EVQLVESGGGLVQPGGSVRLSCVASGIIFRLSALGWTRQGPGKAREWVAGINSDGTTNYADPVKGRFTISRDNAKNTIYLHMDMLKPEDTAVYYCASGKYRGQGTQVTVSSGGGGSGGGGSGGGGSGGGGSGGGGSGGGGSGGGGSEVQLVESGGELVQPGGSLRLSCAASGSILTINAMGWYRQAPGKQRELVVRRTRGGSTTYQDSVKGRFTISADIAKKTMYLQMNSLKPEDTAVYYCMLDDRGGVYWGQGTQVTVSS

SEQ ID NO: 50 - protein, 272 aa, Artificial Sequence
  Sequences of multivalent anti-CXCR2 Nanobodies
EVQLVESGGGLVQPGGSLRLSCVASGSIVRINTMGWYRQTPGKQRELVADITSGGNINYIDAVKGRFTISRDNTKNTVYLQMNSLKPEDTAVYYCNAEIVVLVGVWTQRARTGNYWGQGTQVTVSSGGGGSGGGGSGGGGSGGGGSGGGGSGGGGSGGGGSEVQLVESGGGLVQPGGSVRLSCVASGIIFRLSALGWTRQGPGKAREWVAGINSDGTTNYADPVKGRFTISRDNAKNTIYLHMDMLKPEDTAVYYCASGKYRGQGTQVTVSS

SEQ ID NO: 51 - protein, 272 aa, Artificial Sequence
  Sequences of multivalent anti-CXCR2 Nanobodies
EVQLVESGGGLVQPGGSVRLSCVASGIIFRLSALGWTRQGPGKAREWVAGINSDGTTNYADPVKGRFTISRDNAKNTIYLHMDMLKPEDTAVYYCASGKYRGQGTQVTVSSGGGGSGGGGSGGGGSGGGGSGGGGSGGGGSGGGGSEVQLVESGGGLVQPGGSLRLSCVASGSIVRINTMGWYRQTPGKQRELVADITSGGNINYIDAVKGRFTISRDNTKNTVYLQMNSLKPEDTAVYYCNAEIVVLVGVWTQRARTGNYWGQGTQVTVSS

SEQ ID NO: 52 - protein, 239 aa, Artificial Sequence
  Sequences of multivalent anti-CXCR2 Nanobodies
EVQLVESGGELVQPGGSLRLSCAASGSILTINAMGWYRQAPGKQRELVVRRTRGGSTTYQDSVKGRFTISADIAKKTMYLQMNSLKPEDTAVYYCMLDDRGGVYWGQGTQVTVSSGGGGSGGGSEVQLVESGGELVQPGGSLRLSCAASGSILTINAMGWYRQAPGKQRELVVRRTRGGSTTYQDSVKGRFTISADIAKKTMYLQMNSLKPEDTAVYYCMLDDRGGVYWGQGTQVTVSS

SEQ ID NO: 53 - protein, 274 aa, Artificial Sequence
  Sequences of multivalent anti-CXCR2 Nanobodies
EVQLVESGGGLVQAGESLRLSCAASGSTFDFKVMGWYRQPPGKQREGVAAIRLSGNMHYAESVKGRFTISKANAKNTVYLQMNSLRPEDTAVYYCKVNIRGQDYWGQGTQVTVSSGGGGSGGGGSGGGGSGGGGSGGGGSGGGGSGGGGSEVQLVESGGGLVQAGGSLRLSCAASGRTFSDYAMGWFRQAPGKEREFVAAITWNGGRVFYTASVKGRFTISRDNAKNTMYLQMNSLKPEDTAVYYCAADKDRRTDYLGHPVAYWGQGTQVTVSS

SEQ ID NO: 54 - protein, 272 aa, Artificial Sequence
  Sequences of multivalent anti-CXCR2 Nanobodies
EVQLVESGGGLVQAGESLRLSCAASGSTFDFKVMGWYRQPPGKQREGVAAIRLSGNMHYAESVKGRFTISKANAKNTVYLQMNSLRPEDTAVYYCKVNIRGQDYWGQGTQVTVSSGGGGSGGGGSGGGGSGGGGSGGGGSGGGGSGGGGSEVQLVESGGGLVQPGGSLRLSCVASGRIFSSNAMGWFRQAPGKEREFVAAITWRSGGSAYYADSAKGRFTISRDNAKNTVYLQMNSLKPEDTAVYYCAAGGSSWLSFPPDYWGQGTQVTVSS

SEQ ID NO: 55 - protein, 283 aa, Artificial Sequence
  Sequences of multivalent anti-CXCR2 Nanobodies
EVQLVESGGGLVQAGGSLRLSCAASGRTFSDYAMGWFRQAPGKEREFVAAITWNGGRVFYTASVKGRFTISRDNAKNTMYLQMNSLKPEDTAVYYCAADKDRRTDYLGHPVAYWGQGTQVTVSSGGGGSGGGGSGGGGSGGGGSGGGGSGGGGSGGGGSEVQLVESGGGLVQAGGSLRLSCAASGRTFSDYAMGWFRQAPGKEREFVAAITWNGGRVFYTASVKGRFTISRDNAKNTMYLQMNSLKPEDTAVYYCAADKDRRTDYLGHPVAYWGQGTQVTVSS

SEQ ID NO: 56 - protein, 281 aa, Artificial Sequence
  Sequences of multivalent anti-CXCR2 Nanobodies
EVQLVESGGGLVQAGGSLRLSCAASGRTFSDYAMGWFRQAPGKEREFVAAITWNGGRVFYTASVKGRFTISRDNAKNTMYLQMNSLKPEDTAVYYCAADKDRRTDYLGHPVAYWGQGTQVTVSSGGGGSGGGGSGGGGSGGGGSGGGGSGGGGSGGGGSEVQLVESGGGLVQPGGSLRLSCVASGRIFSSNAMGWFRQAPGKEREFVAAITWRSGGSAYYADSAKGRFTISRDNAKNTVYLQMNSLKPEDTAVYYCAAGGSSWLSFPPDYWGQGTQVTVSS

SEQ ID NO: 57 - protein, 279 aa, Artificial Sequence
  Sequences of multivalent anti-CXCR2 Nanobodies
EVQLVESGGGLVQPGGSLRLSCVASGRIFSSNAMGWFRQAPGKEREFVAAITWRSGGSAYYADSAKGRFTISRDNAKNTVYLQMNSLKPEDTAVYYCAAGGSSWLSFPPDYWGQGTQVTVSSGGGGSGGGGSGGGGSGGGGSGGGGSGGGGSGGGGSEVQLVESGGGLVQPGGSLRLSCVASGRIFSSNAMGWFRQAPGKEREFVAAITWRSGGSAYYADSAKGRFTISRDNAKNTVYLQMNSLKPEDTAVYYCAAGGSSWLSFPPDYWGQGTQVTVSS

SEQ ID NO: 58 - protein, 274 aa, Artificial Sequence
  Sequences of multivalent anti-CXCR2 Nanobodies
EVQLVESGGGLVQAGGSLRLSCAASGRTFSDYAMGWFRQAPGKEREFVAAITWNGGRVFYTASVKGRFTISRDNAKNTMYLQMNSLKPEDTAVYYCAADKDRRTDYLGHPVAYWGQGTQVTVSSGGGGSGGGGSGGGGSGGGGSGGGGSGGGGSGGGGSEVQLVESGGGLVQAGESLRLSCAASGSTFDFKVMGWYRQPPGKQREGVAAIRLSGNMHYAESVKGRFTISKANAKNTVYLQMNSLRPEDTAVYYCKVNIRGQDYWGQGTQVTVSS

SEQ ID NO: 59 - protein, 272 aa, Artificial Sequence
  Sequences of multivalent anti-CXCR2 Nanobodies
EVQLVESGGGLVQPGGSLRLSCVASGRIFSSNAMGWFRQAPGKEREFVAAITWRSGGSAYYADSAKGRFTISRDNAKNTVYLQMNSLKPEDTAVYYCAAGGSSWLSFPPDYWGQGTQVTVSSGGGGSGGGGSGGGGSGGGGSGGGGSGGGGSGGGGSEVQLVESGGGLVQAGESLRLSCAASGSTFDFKVMGWYRQPPGKQREGVAAIRLSGNMHYAESVKGRFTISKANAKNTVYLQMNSLRPEDTAVYYCKVNIRGQDYWGQGTQVTVSS

SEQ ID NO: 60 - protein, 281 aa, Artificial Sequence
  Sequences of multivalent anti-CXCR2 Nanobodies
EVQLVESGGGLVQPGGSLRLSCVASGRIFSSNAMGWFRQAPGKEREFVAAITWRSGGSAYYADSAKGRFTISRDNAKNTVYLQMNSLKPEDTAVYYCAAGGSSWLSFPPDYWGQGTQVTVSSGGGGSGGGGSGGGGSGGGGSGGGGSGGGGSGGGGSEVQLVESGGGLVQAGGSLRLSCAASGRTFSDYAMGWFRQAPGKEREFVAAITWNGGRVFYTASVKGRFTISRDNAKNTMYLQMNSLKPEDTAVYYCAADKDRRTDYLGHPVAYWGQGTQVTVSS

SEQ ID NO: 61 - protein, 281 aa, Artificial Sequence
  Sequences of multivalent anti-CXCR2 Nanobodies
EVQLVESGGGLVQPGGSLRLSCVASGSIVRINTMGWYRQTPGKQRELVADITSGGNINYIDAVKGRFTISRDNTKNTVYLQMNSLKPEDTAVYYCNAEIVVLVGVWTQRARTGNYWGQGTQVTVSSGGGGSGGGGSGGGGSGGGGSGGGGSGGGGSGGGGSEVQLVESGGGLVQAGGSLTLSCAVSGSTFRINTMGWYRRAPGKQRELVAARDRGGYINYVDSVKGRFTVSRDNAKPTMYLQMNSLKPEDTAVYYCHAGTQDRTGRNFDRWGQGTQVTVSS

SEQ ID NO: 62 - protein, 277 aa, Artificial Sequence
  Sequences of multivalent anti-CXCR2 Nanobodies
EVQLVESGGGLVQPGGSLRLSCVASGRIFSSNAMGWFRQAPGKEREFVAAITWRSGGSAYYADSAKGRFTISRDNAKNTVYLQMNSLKPEDTAVYYCAAGGSSWLSFPPDYWGQGTQVTVSSGGGGSGGGGSGGGGSGGGGSGGGGSGGGGSGGGGSEVQLVESGGGLVQAGGSLTLSCAVSGSTFRINTMGWYRRAPGKQRELVAARDRGGYINYVDSVKGRFTVSRDNAKPTMYLQMNSLKPEDTAVYYCHAGTQDRTGRNFDRWGQGTQVTVSS

SEQ ID NO: 63 - protein, 279 aa, Artificial Sequence
  Sequences of multivalent anti-CXCR2 Nanobodies
EVQLVESGGGLVQAGGSLRLSCAASGRTFSDYAMGWFRQAPGKEREFVAAITWNGGRVFYTASVKGRFTISRDNAKNTMYLQMNSLKPEDTAVYYCAADKDRRTDYLGHPVAYWGQGTQVTVSSGGGGSGGGGSGGGGSGGGGSGGGGSGGGGSGGGGSEVQLVESGGGLVQAGGSLTLSCAVSGSTFRINTMGWYRRAPGKQRELVAARDRGGYINYVDSVKGRFTVSRDNAKPTMYLQMNSLKPEDTAVYYCHAGTQDRTGRNFDRWGQGTQVTVSS

SEQ ID NO: 64 - protein, 272 aa, Artificial Sequence
  Sequences of multivalent anti-CXCR2 Nanobodies
EVQLVESGGELVQPGGSLRLSCAASGSILTINAMGWYRQAPGKQRELVVRRTRGGSTTYQDSVKGRFTISADIAKKTMYLQMNSLKPEDTAVYYCMLDDRGGVYWGQGTQVTVSSGGGGSGGGGSGGGGSGGGGSGGGGSGGGGSGGGGSEVQLVESGGGLVQPGGSLRLSCVASGRIFSSNAMGWFRQAPGKEREFVAAITWRSGGSAYYADSAKGRFTISRDNAKNTVYLQMNSLKPEDTAVYYCAAGGSSWLSFPPDYWGQGTQVTVSS

SEQ ID NO: 65 - protein, 274 aa, Artificial Sequence
  Sequences of multivalent anti-CXCR2 Nanobodies
EVQLVESGGELVQPGGSLRLSCAASGSILTINAMGWYRQAPGKQRELVVRRTRGGSTTYQDSVKGRFTISADIAKKTMYLQMNSLKPEDTAVYYCMLDDRGGVYWGQGTQVTVSSGGGGSGGGGSGGGGSGGGGSGGGGSGGGGSGGGGSEVQLVESGGGLVQAGGSLRLSCAASGRTFSDYAMGWFRQAPGKEREFVAAITWNGGRVFYTASVKGRFTISRDNAKNTMYLQMNSLKPEDTAVYYCAADKDRRTDYLGHPVAYWGQGTQVTVSS

SEQ ID NO: 66 - protein, 272 aa, Artificial Sequence
  Sequences of multivalent anti-CXCR2 Nanobodies
EVQLVESGGGLVQPGGSLRLSCVASGRIFSSNAMGWFRQAPGKEREFVAAITWRSGGSAYYADSAKGRFTISRDNAKNTVYLQMNSLKPEDTAVYYCAAGGSSWLSFPPDYWGQGTQVTVSSGGGGSGGGGSGGGGSGGGGSGGGGSGGGGSGGGGSEVQLVESGGELVQPGGSLRLSCAASGSILTINAMGWYRQAPGKQRELVVRRTRGGSTTYQDSVKGRFTISADIAKKTMYLQMNSLKPEDTAVYYCMLDDRGGVYWGQGTQVTVSS

SEQ ID NO: 67 - protein, 274 aa, Artificial Sequence
  Sequences of multivalent anti-CXCR2 Nanobodies
EVQLVESGGGLVQAGGSLRLSCAASGRTFSDYAMGWFRQAPGKEREFVAAITWNGGRVFYTASVKGRFTISRDNAKNTMYLQMNSLKPEDTAVYYCAADKDRRTDYLGHPVAYWGQGTQVTVSSGGGGSGGGGSGGGGSGGGGSGGGGSGGGGSGGGGSEVQLVESGGELVQPGGSLRLSCAASGSILTINAMGWYRQAPGKQRELVVRRTRGGSTTYQDSVKGRFTISADIAKKTMYLQMNSLKPEDTAVYYCMLDDRGGVYWGQGTQVTVSS

SEQ ID NO: 68 - protein, 277 aa, Artificial Sequence
  Sequences of multivalent anti-CXCR2 Nanobodies
EVQLVESGGGLVQAGGSLTLSCAVSGSTFRINTMGWYRRAPGKQRELVAARDRGGYINYVDSVKGRFTVSRDNAKPTMYLQMNSLKPEDTAVYYCHAGTQDRTGRNFDRWGQGTQVTVSSGGGGSGGGGSGGGGSGGGGSGGGGSGGGGSGGGGSEVQLVESGGGLVQPGGSLRLSCVASGRIFSSNAMGWFRQAPGKEREFVAAITWRSGGSAYYADSAKGRFTISRDNAKNTVYLQMNSLKPEDTAVYYCAAGGSSWLSFPPDYWGQGTQVTVSS

SEQ ID NO: 69 - protein, 279 aa, Artificial Sequence
  Sequences of multivalent anti-CXCR2 Nanobodies
EVQLVESGGGLVQAGGSLTLSCAVSGSTFRINTMGWYRRAPGKQRELVAARDRGGYINYVDSVKGRFTVSRDNAKPTMYLQMNSLKPEDTAVYYCHAGTQDRTGRNFDRWGQGTQVTVSSGGGGSGGGGSGGGGSGGGGSGGGGSGGGGSGGGGSEVQLVESGGGLVQAGGSLRLSCAASGRTFSDYAMGWFRQAPGKEREFVAAITWNGGRVFYTASVKGRFTISRDNAKNTMYLQMNSLKPEDTAVYYCAADKDRRTDYLGHPVAYWGQGTQVTVSS

SEQ ID NO: 70 - protein, 30 aa, Artificial Sequence
  fr1
EVQLVESGGGLVQPGGSLRLSCAASGFTFS

SEQ ID NO: 71 - protein, 30 aa, Artificial Sequence
  fr1
EVKLVESGGGLVQAGGSLRLSCALSGRIGS

SEQ ID NO: 72 - protein, 30 aa, Artificial Sequence
  FR1
EVQLVESGGGLVQAGGSLRLSCAASGFTFD

SEQ ID NO: 73 - protein, 30 aa, Artificial Sequence
  FR1
EVQLVESGGGLVQAGGSLSLSCAASGLIFR

SEQ ID NO: 74 - protein, 30 aa, Artificial Sequence
  FR1
EVQLVESGGGLVQAGGSLRLSCAASGRTFS

SEQ ID NO: 75 - protein, 30 aa, Artificial Sequence
  FR1
EVQLVESGGGLVQAGGSLRLSCAASGRSFS

SEQ ID NO: 76 - protein, 30 aa, Artificial Sequence
  FR1
EVQLVESGGGLVQPGGSLRLSCAASGSTLA

SEQ ID NO: 77 - protein, 30 aa, Artificial Sequence
  FR1
KVQLVESGGGLVQAGGSLRLSCAASGRAFN

SEQ ID NO: 78 - protein, 30 aa, Artificial Sequence
  FR1
EVQLVESGGGLVQPGGSVRLSCVASGIIFR

SEQ ID NO: 79 - protein, 30 aa, Artificial Sequence
  FR1
EVQLVESGGGLVQAGESLRLSCAASGSTFD

SEQ ID NO: 80 - protein, 30 aa, Artificial Sequence
  FR1
EVQLVESGGGLVQAGGSLTLSCAVSGSSFR

SEQ ID NO: 81 - protein, 30 aa, Artificial Sequence
  FR1
EVQLVESGGGLVQPGGSLRLSCVASGSIVR

SEQ ID NO: 82 - protein, 30 aa, Artificial Sequence
  FR1
EVQLVESGGGLVQPGGSLRLSCAASGRTFS

SEQ ID NO: 83 - protein, 30 aa, Artificial Sequence; identical to SEQ ID NO: 74
  FR1

SEQ ID NO: 84 - protein, 30 aa, Artificial Sequence
  FR1
EVQLVESGGGLVQPGGSLRLSCVASGRIFS

SEQ ID NO: 85 - protein, 30 aa, Artificial Sequence
  FR1
EVQLVESGGELVQPGGSLRLSCAASGSILT

SEQ ID NO: 86 - protein, 30 aa, Artificial Sequence
  FR1
EVQLVESGGGLVQAGGSLRLTCAASGRIGT

SEQ ID NO: 87 - protein, 30 aa, Artificial Sequence
  FR1
EVQLVESGGGLVQAGGSLRLSCAASGRMGN

SEQ ID NO: 88 - protein, 30 aa, Artificial Sequence
  FR1
EVQLVESGGGLVQAGGSLRLSCAASGTIGT

SEQ ID NO: 89 - protein, 30 aa, Artificial Sequence
  FR1
EVQLVESGGGLVQAGGSLTLSCAVSGSTFR

SEQ ID NO: 90 - protein, 120 aa, Artificial Sequence
  monovalent anti-CXCR2 Nanobodies
EVQLVESGGGLVQAGGSLTLSCAVSGSTFRINTMGWYRRAPGKQRELVAARDRGGYINYVDSVKGRFTVSRDNAKPTMYLQMNSLKPEDTAVYYCHAGTQDRTGRNFDRWGQGTQVTVSS

SEQ ID NO: 91 - protein, 14 aa, Artificial Sequence
  FR2
WVRQAPGKGLDWVS

SEQ ID NO: 92 - protein, 14 aa, Artificial Sequence
  FR2
WYRQVSGQQRELVA

SEQ ID NO: 93 - protein, 14 aa, Artificial Sequence
  FR2
WFRQAPGKERERVS

SEQ ID NO: 94 - protein, 14 aa, Artificial Sequence
  FR2
WYRQAPGRQREWVA

SEQ ID NO: 95 - protein, 14 aa, Artificial Sequence
  FR2
WFRQATGKEREFVA

SEQ ID NO: 96 - protein, 14 aa, Artificial Sequence
  FR2
WLRQAPGKEREFVA

SEQ ID NO: 97 - protein, 14 aa, Artificial Sequence
  FR2
WFRRAPGKEREGIS

SEQ ID NO: 98 - protein, 14 aa, Artificial Sequence
  FR2
WFRQAQGKEREFVA

SEQ ID NO: 99 - protein, 14 aa, Artificial Sequence
  FR2
WTRQGPGKAREWVA

SEQ ID NO: 100 - protein, 14 aa, Artificial Sequence
  FR2
WYRQPPGKQREGVA

SEQ ID NO: 101 - protein, 14 aa, Artificial Sequence
  FR2
WYRRAPGKQRELVA

SEQ ID NO: 102 - protein, 14 aa, Artificial Sequence
  FR2
WYRQTPGKQRELVA

SEQ ID NO: 103 - protein, 14 aa, Artificial Sequence
  FR2
WFRQAPGKERAFVA

SEQ ID NO: 104 - protein, 14 aa, Artificial Sequence
  FR2
WFRQAPGKEREFVA

SEQ ID NO: 105 - protein, 14 aa, Artificial Sequence
  FR2
WFRQAPGKEREFVA

SEQ ID NO: 106 - protein, 14 aa, Artificial Sequence
  FR2
WYRQAPGKQRELVV

SEQ ID NO: 107 - protein, 14 aa, Artificial Sequence
  FR2
WYRQAPGKQRELVA

SEQ ID NO: 108 - protein, 14 aa, Artificial Sequence
  FR2
WYRQAPGKERELVA

SEQ ID NO: 109 - protein, 14 aa, Artificial Sequence
  FR2
WYRQAPGKQRELVA

SEQ ID NO: 110 - protein, 14 aa, Artificial Sequence
  FR2
WYRRAPGKQRELVA

SEQ ID NO: 111 - protein, 32 aa, Artificial Sequence
  FR3
RFTISRDNNKNTLYLQMNSLKPEDTALYYCAT

SEQ ID NO: 112 - protein, 32 aa, Artificial Sequence
  FR3
RFTISRDNGKNTVYLQMDSLKPEDTAVYYCYA

SEQ ID NO: 113 - protein, 32 aa, Artificial Sequence
  FR3
RFTISSDNAKNTVYLQMNNLKPEDTAVYYCAA

SEQ ID NO: 114 - protein, 32 aa, Artificial Sequence
  FR3
RFTISRNNAENTWYLQMNSLKPEDTAIYYCNT

SEQ ID NO: 115 - protein, 32 aa, Artificial Sequence
  FR3
RFTISRDNAKNTVYLQMNSLKPRDTAVYYCAA

SEQ ID NO: 116 - protein, 32 aa, Artificial Sequence
  FR3
RFTISRDNAKNTVSLQMNSLKPQDTAVYYCAA

SEQ ID NO: 117 - protein, 32 aa, Artificial Sequence
  FR3
RFTISRDNAKNTVYLQMNSLKPEDTAVYYCAA

SEQ ID NO: 118 - protein, 32 aa, Artificial Sequence
  FR3
RFTISRDNAKNTVYLHMNSLKPEDTAVYYCAA

SEQ ID NO: 119 - protein, 32 aa, Artificial Sequence
  FR3
RFTISRDNAKNTIYLHMDMLKPEDTAVYYCAS

SEQ ID NO: 120 - protein, 32 aa, Artificial Sequence
  FR3
RFTISKANAKNTVYLQMNSLRPEDTAVYYCKV

SEQ ID NO: 121 - protein, 32 aa, Artificial Sequence
  FR3
RFTVSRDNAKPTMYLQMNSLKPEDTAVYYCHA

SEQ ID NO: 122 - protein, 32 aa, Artificial Sequence
  FR3
RFTISRDNTKNTVYLQMNSLKPEDTAVYYCNA

SEQ ID NO: 123 - protein, 32 aa, Artificial Sequence
  FR3
RFTISRDVAKKTLYLQMNSLKPEDTAVYYCAA

SEQ ID NO: 124 - protein, 32 aa, Artificial Sequence
  FR3
RFTISRDNAKNTMYLQMNSLKPEDTAVYYCAA

SEQ ID NO: 125 - protein, 32 aa, Artificial Sequence; identical to SEQ ID NO: 117
  FR3

SEQ ID NO: 126 - protein, 32 aa, Artificial Sequence
  FR3
RFTISADIAKKTMYLQMNSLKPEDTAVYYCML

SEQ ID NO: 127 - protein, 32 aa, Artificial Sequence
  FR3
RFTISRDNAKNTVYLQMNSLKPEDTAVYYYNV

SEQ ID NO: 128 - protein, 32 aa, Artificial Sequence
  FR3
RFTIARDNILNTAYLQMNDLKPEDTAVYYYNV

SEQ ID NO: 129 - protein, 32 aa, Artificial Sequence
  FR3
RFTIGRDNAKNTAYLQMNNLKPEDTAVYYYNI

SEQ ID NO: 130 - protein, 32 aa, Artificial Sequence; identical to SEQ ID NO: 121
  FR3

SEQ ID NO: 131 - protein, 11 aa, Artificial Sequence
  FR4
WGQGTQVTVSS

SEQ ID NO: 132 - protein, 11 aa, Artificial Sequence
  FR4
RGQGTQVTVSS

SEQ ID NO: 133 - protein, 11 aa, Artificial Sequence
  FR4
WGQGTQVTVSS

SEQ ID NO: 134 - protein, 5 aa, Artificial Sequence
  CDR1
DYAIG

SEQ ID NO: 135 - protein, 5 aa, Artificial Sequence
  CDR1
LSGMA

SEQ ID NO: 136 - protein, 5 aa, Artificial Sequence
  CDR1
NYAMG

SEQ ID NO: 137 - protein, 5 aa, Artificial Sequence
  CDR1
RSAMG

SEQ ID NO: 138 - protein, 5 aa, Artificial Sequence
  CDR1
YYTVG

SEQ ID NO: 139 - protein, 5 aa, Artificial Sequence
  CDR1
YYVMA

SEQ ID NO: 140 - protein, 5 aa, Artificial Sequence
  CDR1
LSALG

SEQ ID NO: 141 - protein, 5 aa, Artificial Sequence
  CDR1
FKVMG

SEQ ID NO: 142 - protein, 5 aa, Artificial Sequence
  CDR1
INTMG

SEQ ID NO: 143 - protein, 5 aa, Artificial Sequence
  CDR1
INTMG

SEQ ID NO: 144 - protein, 5 aa, Artificial Sequence
  CDR1
SLSMG

SEQ ID NO: 145 - protein, 5 aa, Artificial Sequence
  CDR1
DYAMG

SEQ ID NO: 146 - protein, 5 aa, Artificial Sequence
  CDR1
SNAMG

SEQ ID NO: 147 - protein, 5 aa, Artificial Sequence
  CDR1
INAMG

SEQ ID NO: 148 - protein, 5 aa, Artificial Sequence
  CDR1
INAMG

SEQ ID NO: 149 - protein, 5 aa, Artificial Sequence
  CDR1
INAMG

SEQ ID NO: 150 - protein, 5 aa, Artificial Sequence
  CDR1
IRAMG

SEQ ID NO: 151 - protein, 5 aa, Artificial Sequence
  CDR1
INTMG

SEQ ID NO: 152 - protein, 17 aa, Artificial Sequence
  CDR2
AINAGGDSTYYADPVKG

SEQ ID NO: 153 - protein, 16 aa, Artificial Sequence
  CDR2
VSRSGGSTDIADSVKG

SEQ ID NO: 154 - protein, 17 aa, Artificial Sequence
  CDR2
CISGSDGSTYYADSVKG

SEQ ID NO: 155 - protein, 16 aa, Artificial Sequence
  CDR2
VLTKDGTLHYADPVKG

SEQ ID NO: 156 - protein, 17 aa, Artificial Sequence
  CDR2
AINKSGGNTHYAGSVKG

SEQ ID NO: 157 - protein, 17 aa, Artificial Sequence
  CDR2
GISWGGDNSYYADSVKG

SEQ ID NO: 158 - protein, 17 aa, Artificial Sequence
  CDR2
CISSSDGSTYYADSVKG

SEQ ID NO: 159 - protein, 17 aa, Artificial Sequence
  CDR2
AISTRGSMTKYSDSVQG

SEQ ID NO: 160 - protein, 16 aa, Artificial Sequence
  CDR2
GINSDGTTNYADPVKG

SEQ ID NO: 161 - protein, 16 aa, Artificial Sequence
  CDR2
AIRLSGNMHYAESVKG

SEQ ID NO: 162 - protein, 16 aa, Artificial Sequence
  CDR2
ARDRGGYINYVDSVKG

SEQ ID NO: 163 - protein, 16 aa, Artificial Sequence
  CDR2
DITSGGNINYIDAVKG

SEQ ID NO: 164 - protein, 17 aa, Artificial Sequence
  CDR2
ALTRNGGYRYYADSVKG

SEQ ID NO: 165 - protein, 17 aa, Artificial Sequence
  CDR2
AITWNGGRVFYTASVKG

SEQ ID NO: 166 - protein, 18 aa, Artificial Sequence
  CDR2
AITWRSGGSAYYADSAKG

SEQ ID NO: 167 - protein, 16 aa, Artificial Sequence
  CDR2
RRTRGGSTTYQDSVKG

SEQ ID NO: 168 - protein, 16 aa, Artificial Sequence
  CDR2
VITSGGRIDYADSVKG

SEQ ID NO: 169 - protein, 16 aa, Artificial Sequence
  CDR2
KITRGGAITYADSVKG

SEQ ID NO: 170 - protein, 16 aa, Artificial Sequence
  CDR2
LITSTGRINYADSVKG

SEQ ID NO: 171 - protein, 16 aa, Artificial Sequence
  CDR2
ARDRGGYINYVDSVKG

SEQ ID NO: 172 - protein, 10 aa, Artificial Sequence
  CDR3
VRGTARDLDY

SEQ ID NO: 173 - protein, 15 aa, Artificial Sequence
  CDR3
HTSSYSNWRVYNNDY

SEQ ID NO: 174 - protein, 17 aa, Artificial Sequence
  CDR3
YWGLTLRLWMPPHRYDY

SEQ ID NO: 175 - protein, 3 aa, Artificial Sequence
  CDR3
GRY

SEQ ID NO: 176 - protein, 9 aa, Artificial Sequence
  CDR3
SRTNPKPDY

SEQ ID NO: 177 - protein, 13 aa, Artificial Sequence
  CDR3
RYRGGAAVAGWEY

SEQ ID NO: 178 - protein, 15 aa, Artificial Sequence
  CDR3
DRRTDCKKGRVGSGS

SEQ ID NO: 179 - protein, 16 aa, Artificial Sequence
  CDR3
DPRGSSWSFSSGGYDY

SEQ ID NO: 180 - protein, 3 aa, Artificial Sequence
  CDR3
GKY

SEQ ID NO: 181 - protein, 7 aa, Artificial Sequence
  CDR3
NIRGQDY

SEQ ID NO: 182 - protein, 12 aa, Artificial Sequence
  CDR3
GTQDRTGRNFDH

SEQ ID NO: 183 - protein, 18 aa, Artificial Sequence
  CDR3
EIVVLVGVWTQRARTGNY

SEQ ID NO: 184 - protein, 15 aa, Artificial Sequence
  CDR3
DSLSGSDYLGTNLDY

SEQ ID NO: 185 - protein, 15 aa, Artificial Sequence
  CDR3
DKDRRTDYLGHPVAY

SEQ ID NO: 186 - protein, 12 aa, Artificial Sequence
  CDR3
GGSSWLSFPPDY

SEQ ID NO: 187 - protein, 7 aa, Artificial Sequence
  CDR3
DDRGGVY

SEQ ID NO: 188 - protein, 8 aa, Artificial Sequence
  CDR3
ETVVGAVY

SEQ ID NO: 189 - protein, 8 aa, Artificial Sequence
  CDR3
DGGPSQNY

SEQ ID NO: 190 - protein, 7 aa, Artificial Sequence
  CDR3
ETLRRNY

SEQ ID NO: 191 - protein, 12 aa, Artificial Sequence
  CDR3
GTQDRTGRNFDR

SEQ ID NO: 192 - DNA, 357 bp, Artificial Sequence
  NUCLEIC ACID ENCODING MONOVALENT NANOBODY
gaggtgcagctggtggagtctgggggaggcttggtgcagcctggggggtctctgagactctcctgtgcagcctctggattcaccttcagtacctactggatgtattgggtccgtcaggctccagggaaggggctcgactgggtctcagctattaatgctggtggtgatagcacatactatgcagaccccgtgaagggccgattcaccatctccagagacaacaacaagaacacgctgtatctgcagatgaacagcctgaaacctgaggacacggccctgtattactgtgcgaccgtacgaggcacagctcgtgacttggactactggggccaggggacccaggtcaccgtctcctca

SEQ ID NO: 193 - DNA, 369 bp, Artificial Sequence
  NUCLEIC ACID ENCODING MONOVALENT NANOBODY
gaggtgaagctggtggagtctgggggaggcttggtgcaggctggggggtctctgagactctcctgtgcactctctggaaggatcggcagtatcaacgccatgggctggtatcgccaggtttcaggacaacagcgcgagttggtcgcagtaagcaggagcggaggtagcacagacattgctgactccgtgaagggccgattcaccatctccagagacaacggcaagaacacagtgtatctgcagatggacagcctgaaacctgaggacacggccgtctattactgttatgctcatacttcaagctatagtaattggcgagtctacaataacgactactggggccaggggacccaggtcaccgtctcctca

SEQ ID NO: 194 - DNA, 348 bp, Artificial Sequence
  NUCLEIC ACID ENCODING MONOVALENT NANOBODY
gaggtgcagctggtggagtctgggggaggcttggtgcaggctggggggtctctgagacttacctgtgcagcctctggacgcatcggcactatcaatgccatgggctggtaccgccaggctccagggaagcagcgcgagttggtcgcagttattactagtggtggtaggatagactatgcagactccgtgaagggccgattcaccatctccagagacaatgccaagaacacggtgtatctgcaaatgaacagcctgaaacctgaggacacggccgtctattactataatgtagaaacggtagtgggtgccgtctactggggccaggggacccaggtcaccgtctcctca

SEQ ID NO: 195 - DNA, 348 bp, Artificial Sequence
  NUCLEIC ACID ENCODING MONOVALENT NANOBODY
gaggtgcagctggtggagtctgggggaggcttggtgcaggctggggggtctctgagactctcctgtgcagcctctggaaggatgggcaatatcaatgccatgggctggtatcgccaggctccagggaaggagcgcgagttggtcgcaaaaattactaggggtggtgcgataacctatgcagactccgtgaagggccgattcaccatcgccagagacaatattctgaacacggcgtatctgcaaatgaacgacctgaaacctgaggacacggccgtctattattataatgtagatggggggcccagtcaaaactactggggccaggggacccaggtcaccgtctcctca

SEQ ID NO: 196 - DNA, 378 bp, Artificial Sequence
  NUCLEIC ACID ENCODING MONOVALENT NANOBODY
gaggtgcagctggtggagtctgggggaggcttggtgcaggctggggggtctctgagactctcctgtgcagcctctggattcactttcgatgattatgccataggctggttccgccaggccccagggaaggagcgtgagagggtctcatgtattagtggtagtgatggtagcacatactatgcagactccgtcaagggccgattcaccatctccagtgacaacgccaagaacacggtgtatctgcaaatgaacaacctgaaacccgaggacacggccgtttattattgtgcagcatattggggactaacgctcaggctatggatgcccccccaccggtatgactactggggccaggggacccaggtcaccgtctcctca

SEQ ID NO: 197 - DNA, 333 bp, Artificial Sequence
  NUCLEIC ACID ENCODING MONOVALENT NANOBODY
gaggtgcagctggtggagtctgggggaggcttggtgcaggctggggggtctctgagcctctcctgtgcagcctctggacttatcttcagactcagtggcatggcctggtatcgccaggctccggggaggcagcgcgagtgggtcgcagtgcttaccaaagatggtaccctacactatgcagaccccgtgaagggccgattcaccatctccagaaacaacgccgagaacacgtggtatctgcaaatgaacagcctgaaacctgaggacacagccatctattactgtaatacgggccgttactggggccaggggacccaggtcaccgtctcctca

SEQ ID NO: 198 - DNA, 345 bp, Artificial Sequence
  NUCLEIC ACID ENCODING MONOVALENT NANOBODY
gaggtgcagctggtggagtctgggggaggcttggtgcaggctggggggtcactgagactctcctgtgcagcctctggaaccatcggcacgatcagagccatgggctggtaccgccaggctccagggaagcagcgcgagttggtcgcattgattactagtactggtaggataaactatgcagactccgtgaagggccgattcaccattggaagagacaatgccaagaacacggcgtatctgcaaatgaacaacctgaaacctgaggacacggccgtctattactataatatcgaaacactacgacgtaactactggggccaggggacccaggtcaccgtctcctca

SEQ ID NO: 199 - DNA, 354 bp, Artificial Sequence
  NUCLEIC ACID ENCODING MONOVALENT NANOBODY
gaggtgcagctggtggagtctgggggaggattggtgcaggctggggggtctctgagactctcctgtgcagcctctggacgcacctttagtaactatgccatgggctggttccgccaggccacagggaaggagcgtgagtttgtagcagctattaacaagagtggtgggaacacacactatgcaggctccgtgaagggccgattcaccatctccagagacaacgccaagaacacggtgtatctgcaaatgaacagcctgaaacctagggacacggccgtttattactgtgcagcgtcgcggactaaccctaagcctgactactggggccaggggacccaggtcaccgtctcctca

SEQ ID NO: 200 - DNA, 366 bp, Artificial Sequence
  NUCLEIC ACID ENCODING MONOVALENT NANOBODY
gaggtgcagctggtggagtctgggggaggattggtgcaggctgggggctctctgagactctcctgtgcagcctctggacgctccttcagtcgcagtgccatgggctggctccgccaggctccagggaaggagcgtgaatttgtagcaggtattagctggggtggtgataactcatactatgcagactccgtgaagggccgattcaccatctccagagacaacgccaagaacaccgtgtctctacaaatgaacagcctgaaacctcaggacacggccgtttattactgtgcagcaagataccggggaggcgcggcagtagctggttgggagtactggggccaggggacccaggtcaccgtctcctca

SEQ ID NO: 201 - DNA, 372 bp, Artificial Sequence
  NUCLEIC ACID ENCODING MONOVALENT NANOBODY
gaggtgcagctggtggagtctgggggaggcttggtgcagcctggggggtctctgagactctcctgtgcagcctccggatccactttggcctattataccgtaggctggttccgccgggccccagggaaggagcgcgaggggatctcatgtattagtagtagtgatggtagcacatactatgcagactccgtgaagggccgattcaccatctccagagacaatgccaagaatacggtgtatctgcaaatgaacagcctgaaacctgaggacacggccgtttattactgtgcggctgacagacgtaccgactgtaaaaagggtagagtcggttctggttcctggggccaggggacccaggtcaccgtctcctca

SEQ ID NO: 202 - DNA, 375 bp, Artificial Sequence
  NUCLEIC ACID ENCODING MONOVALENT NANOBODY
aaggtgcagctggtggagtctgggggagggctggtgcaggctgggggctctctgagactctcctgtgcagcctccggacgcgccttcaattactatgtcatggcctggttccgccaggctcaagggaaggagcgtgagtttgtagcagctattagcacgcgtggtagtatgacaaagtattcagactccgtgcagggccggttcaccatctccagagacaacgccaagaacacggtgtatctgcacatgaacagcctgaaacctgaggatacggccgtttattactgtgcagcagaccctcgcggcagtagctggtcattttcgtccgggggttatgactactggggccaggggacccaggtcaccgtctcctca

SEQ ID NO: 203 - DNA, 333 bp, Artificial Sequence
  NUCLEIC ACID ENCODING MONOVALENT NANOBODY
gaggtgcagctggtggagtctgggggaggcttggtgcagcctggggggtctgtgagactctcctgtgtagcctctggaatcatcttcagactcagtgcgttgggttggacacgccagggtccaggaaaggcgcgcgagtgggtcgcaggtattaacagtgatggtacgaccaactacgccgaccccgtgaagggccgattcaccatctccagagacaacgccaagaacacgatatatctgcacatggacatgctgaaacctgaggatacggccgtctattactgtgcctccggaaagtaccggggccaggggacccaggtcaccgtctcctca

SEQ ID NO: 204 - DNA, 345 bp, Artificial Sequence
  NUCLEIC ACID ENCODING MONOVALENT NANOBODY
gaggtgcagctggtggagtctgggggaggcttggtgcaggctggggagtctctgagactctcctgtgcagcctctggaagcaccttcgatttcaaagtcatgggctggtaccgccagcctccagggaagcagcgcgagggggtcgcagcgattaggcttagtggtaacatgcactatgcagagtccgtgaagggccgattcaccatctccaaagccaacgccaagaacacagtgtatctgcaaatgaacagcctgagacctgaggacacggccgtctattactgtaaggtgaacattcggggccaggactactggggccaggggacccaggtcaccgtctcctca

SEQ ID NO: 205 - DNA, 360 bp, Artificial Sequence
  NUCLEIC ACID ENCODING MONOVALENT NANOBODY
gaggtgcagctggtggagtctgggggaggcttggtgcaggctggggggtctctgacgctctcctgtgcagtctctggaagctccttcagaatcaataccatgggctggtaccgccgggctccagggaagcagcgcgagttggtcgcagctcgtgatagaggtggttacataaactatgtagattccgtgaagggccgattcaccgtctccagagacaacgccaagcccacaatgtatctgcaaatgaacagcctgaaacctgaggacacggccgtctattattgtcatgccgggacccaagatcggacgggtcggaatttcgaccactggggccaggggacccaggtcaccgtctcctca

SEQ ID NO: 206 - DNA, 378 bp, Artificial Sequence
  NUCLEIC ACID ENCODING MONOVALENT NANOBODY
gaggtgcagctggtggagtctgggggaggcttggtgcagcctggggggtctctgagactctcctgtgtagcctctggaagcatcgtcagaattaataccatgggctggtaccgccagactccagggaagcagcgcgagttggtcgcagatattaccagtggtggtaacataaactatatagacgccgtgaagggccgattcaccatctccagagacaacaccaagaacacggtgtatctgcaaatgaacagcctgaaacctgaggacacggccgtctattactgtaatgcagagatcgttgttctggtgggagtttggacccagcgtgcgcggaccggcaactactggggccaggggacccaggtcaccgtctcctca

SEQ ID NO: 207 - DNA, 372 bp, Artificial Sequence
  NUCLEIC ACID ENCODING MONOVALENT NANOBODY
gaggtgcagctggtggagtctgggggaggattggtgcagcctggggggtctctgagactctcctgtgcagcctctggacgcacgttcagtagcttgtccatgggctggttccgccaggctccggggaaggagcgtgcctttgtagcagcgcttactcgaaatggtggttacagatactatgcagactccgtgaagggccgattcaccatctccagagacgtcgccaagaagaccttatatctgcaaatgaacagcctgaaacctgaggacacggccgtctattactgtgcagcagatagtcttagtggtagtgactacttaggaaccaacctagactactggggccaggggacccaggtcaccgtctcctca

SEQ ID NO: 208 - DNA, 372 bp, Artificial Sequence
  NUCLEIC ACID ENCODING MONOVALENT NANOBODY
gaggtgcagctggtggagtctgggggaggattggtgcaggctgggggctctctgagactctcctgtgcagcctctggacgcaccttcagtgactatgccatgggctggttccgccaggctccagggaaggagcgtgagtttgtagcagctattacgtggaatggtggtagagtattttatactgcctccgtgaagggccgattcaccatctccagagacaacgccaagaacacgatgtatctgcaaatgaacagcctgaaacctgaggacacggccgtttattactgtgcagcagataaagacagacgtactgactatctagggcaccccgttgcctactggggccaggggacccaggtcaccgtctcctca

SEQ ID NO: 209 - DNA, 366 bp, Artificial Sequence
  NUCLEIC ACID ENCODING MONOVALENT NANOBODY
gaggtgcagctggtggagtctgggggaggattggtgcagcctgggggctctctgagactctcctgtgtagcctctggacgcatcttcagtagcaatgccatgggctggttccgccaggctccagggaaggagcgtgagtttgtagcggccattacctggaggagtggcggtagcgcgtactatgcagactccgcgaagggccgattcaccatctccagagacaacgccaagaacacggtgtatttgcaaatgaacagcctgaaacctgaggacacggccgtttattattgtgcagctggtggtagttcctggttaagttttccgccggactactggggccaggggacccaggtcaccgtctcctca

SEQ ID NO: 210 - DNA, 345 bp, Artificial Sequence
  NUCLEIC ACID ENCODING MONOVALENT NANOBODY
gaggtgcagctggtggagtctgggggagagttggtgcagccgggggggtctctgagactctcctgtgcagcctctggaagcatcttaactatcaatgccatgggctggtaccgccaggctccagggaagcagcgcgagttggtagtccgtaggactaggggtggtagtacaacgtatcaagactccgtgaagggccgattcaccatctccgcagacattgccaagaaaacgatgtatctccaaatgaacagcctgaaacctgaagacacggccgtctattactgtatgctagatgaccgtgggggtgtctactggggtcaggggacccaggtcaccgtctcctca

SEQ ID NO: 211 - DNA, 360 bp, Artificial Sequence
  NUCLEIC ACID ENCODING MONOVALENT NANOBODY
gaggtgcagctggtggagtctgggggaggcttggtgcaggctggggggtctctgacgctctcctgtgcagtctctggaagcaccttcagaatcaataccatgggctggtaccgccgggctccagggaagcagcgcgagttggtcgcagctcgtgatagaggtggttacataaactatgtagattccgtgaagggccgattcaccgtctccagagacaacgccaagcccacaatgtatctgcaaatgaacagcctgaaacctgaggacacggccgtctattattgtcatgccgggacccaagatcggacgggtcggaatttcgaccgctggggccaggggacccaggtcaccgtctcctca

SEQ ID NO: 212 - protein, 109 aa, Homo sapiens
EVQLLESGGGLVQPGGSLRLSCAASGFTFSSYAMSWVRQAPGKGLEWVSAISGSGGSTYYADSVKGRFTISRDNSKNTLYLQMNSLRAEDTAVYYCAKWGQGTLVTVSS

SEQ ID NO: 213 - protein, 115 aa, Artificial Sequence
  Amino acid sequences of sequence-optimised variants
EVQLLESGGGLVQPGGSLRLSCAASGSILTINAMGWYRQAPGKQRELVVRRTRGGSTTYQDSVKGRFTISADISKKTMYLQMNSLRPEDTAVYYCLLDDRGGVYWGQGTLVTVSS

SEQ ID NO: 214 - protein, 115 aa, Artificial Sequence
  Amino acid sequences of sequence-optimised variants
EVQLLESGGGLVQPGGSLRLSCAASGSILTINAMGWYRQAPGKQRELVVRRTRGGSTTYQDSVKGRFTISADISKNTMYLQMNSLRPEDTAVYYCLLDDRGGVYWGQGTLVTVSS

SEQ ID NO: 215 - protein, 126 aa, Artificial Sequence
  Amino acid sequences of sequence-optimised variants
EVQLLESGGGLVQPGGSLRLSCAASGSIVRINTMGWYRQAPGKQRELVADITSGGNINYADSVKGRFTISRDNSKNTVYLQMNSLRPEDTAVYYCNAEIVVLVGVWTQRARTGNYWGQGTLVTVSS

SEQ ID NO: 216 - protein, 115 aa, Artificial Sequence
  Amino acid sequences of sequence-optimised variants
EVQLLESGGGLVQPGGSLRLSCAASGSTFDFKVMGWYRQAPGKQREGVAAIRLSGNRHYAESVKGRFTISRANSKNTVYLQMNSLRPEDTAVYYCKVNIRGQDYWGQGTLVTVSS

SEQ ID NO: 217 - protein, 122 aa, Artificial Sequence
  Amino acid sequences of sequence-optimised variants
EVQLLESGGGLVQPGGSLRLSCAASGRIFSSNAMGWFRQAPGKEREFVAAITWRSGGSAYYADSVKGRFTISRDNSKNTVYLQMNSLRPEDTAVYYCAAGGSSWLSFPPDYWGQGTLVTVSS

SEQ ID NO: 218 - protein, 124 aa, Artificial Sequence
  Amino acid sequences of sequence-optimised variants
EVQLLESGGGLVQPGGSLRLSCAASGRTFSDYAMGWFRQAPGKEREFVAAITWNGGRVFYTASVKGRFTISRDNSKNTLYLQMNSLRPEDTAVYYCAADKDRRTDYLGHPVAYWGQGTLVTVSS

SEQ ID NO: 219 - protein, 120 aa, Artificial Sequence
  Amino acid sequences of sequence-optimised variants
EVQLLESGGGLVQPGGSLRLSCAVSGSTFRINTMGWYRQAPGKQRELVAARDRGGYINYVDSVKGRFTISRDNSKPTMYLQMNSLRPEDTAVYYCHAGTQDRTGRNFDRWGQGTLVTVSS

SEQ ID NO: 220 - protein, 35 aa, Artificial Sequence
  PEPTIDE LINKER
GGGGSGGGGSGGGGSGGGGSGGGGSGGGGSGGGGS

SEQ ID NO: 221 - protein, 272 aa, Artificial Sequence
  amino acid sequences of sequence-optimised biparatopic
EVQLLESGGGLVQPGGSLRLSCAASGSTFDFKVMGWYRQAPGKQREGVAAIRLSGNRHYAESVKGRFTISRANSKNTVYLQMNSLRPEDTAVYYCKVNIRGQDYWGQGTLVTVSSGGGGSGGGGSGGGGSGGGGSGGGGSGGGGSGGGGSEVQLLESGGGLVQPGGSLRLSCAASGRIFSSNAMGWFRQAPGKEREFVAAITWRSGGSAYYADSVKGRFTISRDNSKNTVYLQMNSLRPEDTAVYYCAAGGSSWLSFPPDYWGQGTLVTVSS

SEQ ID NO: 222 - protein, 274 aa, Artificial Sequence
  amino acid sequences of sequence-optimised biparatopic
EVQLLESGGGLVQPGGSLRLSCAASGSTFDFKVMGWYRQAPGKQREGVAAIRLSGNRHYAESVKGRFTISRANSKNTVYLQMNSLRPEDTAVYYCKVNIRGQDYWGQGTLVTVSSGGGGSGGGGSGGGGSGGGGSGGGGSGGGGSGGGGSEVQLLESGGGLVQPGGSLRLSCAASGRTFSDYAMGWFRQAPGKEREFVAAITWNGGRVFYTASVKGRFTISRDNSKNTLYLQMNSLRPEDTAVYYCAADKDRRTDYLGHPVAYWGQGTLVTVSS

SEQ ID NO: 223 - protein, 277 aa, Artificial Sequence
  amino acid sequences of sequence-optimised biparatopic
EVQLLESGGGLVQPGGSLRLSCAVSGSTFRINTMGWYRQAPGKQRELVAARDRGGYINYVDSVKGRFTISRDNSKPTMYLQMNSLRPEDTAVYYCHAGTQDRTGRNFDRWGQGTLVTVSSGGGGSGGGGSGGGGSGGGGSGGGGSGGGGSGGGGSEVQLLESGGGLVQPGGSLRLSCAASGRIFSSNAMGWFRQAPGKEREFVAAITWRSGGSAYYADSVKGRFTISRDNSKNTVYLQMNSLRPEDTAVYYCAAGGSSWLSFPPDYWGQGTLVTVSS

SEQ ID NO: 224 - protein, 279 aa, Artificial Sequence
  amino acid sequences of sequence-optimised biparatopic
EVQLLESGGGLVQPGGSLRLSCAVSGSTFRINTMGWYRQAPGKQRELVAARDRGGYINYVDSVKGRFTISRDNSKPTMYLQMNSLRPEDTAVYYCHAGTQDRTGRNFDRWGQGTLVTVSSGGGGSGGGGSGGGGSGGGGSGGGGSGGGGSGGGGSEVQLLESGGGLVQPGGSLRLSCAASGRTFSDYAMGWFRQAPGKEREFVAAITWNGGRVFYTASVKGRFTISRDNSKNTLYLQMNSLRPEDTAVYYCAADKDRRTDYLGHPVAYWGQGTLVTVSS

SEQ ID NO: 225 - protein, 422 aa, Artificial Sequence
  amino acid sequences of sequence-optimised biparatopic
EVQLLESGGGLVQPGGSLRLSCAASGSTFDFKVMGWYRQAPGKQREGVAAIRLSGNRHYAESVKGRFTISRANSKNTVYLQMNSLRPEDTAVYYCKVNIRGQDYWGQGTLVTVSSGGGGSGGGGSGGGGSGGGGSGGGGSGGGGSGGGGSEVQLLESGGGLVQPGGSLRLSCAASGRIFSSNAMGWFRQAPGKEREFVAAITWRSGGSAYYADSVKGRFTISRDNSKNTVYLQMNSLRPEDTAVYYCAAGGSSWLSFPPDYWGQGTLVTVSSGGGGSGGGGSGGGGSGGGGSGGGGSGGGGSGGGGSEVQLVESGGGLVQPGNSLRLSCAASGFTFSSFGMSWVRQAPGKGLEWVSSISGSGSDTLYADSVKGRFTISRDNAKTTLYLQMNSLRPEDTAVYYCTIGGSLSRSSQGTLVTVSS

SEQ ID NO: 226 - protein, 426 aa, Artificial Sequence
  amino acid sequences of sequence-optimised biparatopic
EVQLLESGGGLVQPGGSLRLSCAASGSTFDFKVMGWYRQAPGKQREGVAAIRLSGNRHYAESVKGRFTISRANSKNTVYLQMNSLRPEDTAVYYCKVNIRGQDYWGQGTLVTVSSGGGGSGGGGSGGGGSGGGGSGGGGSGGGGSGGGGSEVQLLESGGGLVQPGGSLRLSCAASGSIVRINTMGWYRQAPGKQRELVADITSGGNINYADSVKGRFTISRDNSKNTVYLQMNSLRPEDTAVYYCNAEIVVLVGVWTQRARTGNYWGQGTLVTVSSGGGGSGGGGSGGGGSGGGGSGGGGSGGGGSGGGGSEVQLVESGGGLVQPGNSLRLSCAASGFTFSSFGMSWVRQAPGKGLEWVSSISGSGSDTLYADSVKGRFTISRDNAKTTLYLQMNSLRPEDTAVYYCTIGGSLSRSSQGTLVTVSS

SEQ ID NO: 227 - protein, 424 aa, Artificial Sequence
  amino acid sequences of sequence-optimised biparatopic
EVQLLESGGGLVQPGGSLRLSCAASGSTFDFKVMGWYRQAPGKQREGVAAIRLSGNRHYAESVKGRFTISRANSKNTVYLQMNSLRPEDTAVYYCKVNIRGQDYWGQGTLVTVSSGGGGSGGGGSGGGGSGGGGSGGGGSGGGGSGGGGSEVQLLESGGGLVQPGGSLRLSCAASGRTFSDYAMGWFRQAPGKEREFVAAITWNGGRVFYTASVKGRFTISRDNSKNTLYLQMNSLRPEDTAVYYCAADKDRRTDYLGHPVAYWGQGTLVTVSSGGGGSGGGGSGGGGSGGGGSGGGGSGGGGSGGGGSEVQLVESGGGLVQPGNSLRLSCAASGFTFSSFGMSWVRQAPGKGLEWVSSISGSGSDTLYADSVKGRFTISRDNAKTTLYLQMNSLRPEDTAVYYCTIGGSLSRSSQGTLVTVSS

SEQ ID NO: 228 - protein, 115 aa, Artificial Sequence [sequence omitted]

SEQ ID NO: 229 - protein, 30 aa, Artificial Sequence
  FR1
EVQLLESGGGLVQPGGSLRLSCAASGSILT

SEQ ID NO: 230 - protein, 30 aa, Artificial Sequence
  FR1
EVQLLESGGGLVQPGGSLRLSCAASGSIVR

SEQ ID NO: 231 - protein, 30 aa, Artificial Sequence
  FR1
EVQLLESGGGLVQPGGSLRLSCAASGSTFD

SEQ ID NO: 232 - protein, 30 aa, Artificial Sequence
  FR1
EVQLLESGGGLVQPGGSLRLSCAASGRIFS

SEQ ID NO: 233 - protein, 30 aa, Artificial Sequence
  FR1
EVQLLESGGGLVQPGGSLRLSCAASGRTFS

SEQ ID NO: 234 - protein, 30 aa, Artificial Sequence
  FR1
EVQLLESGGGLVQPGGSLRLSCAVSGSTFR

SEQ ID NO: 235 - protein, 16 aa, Artificial Sequence
  CDR2
DITSGGNINYADSVKG

SEQ ID NO: 236 - protein, 16 aa, Artificial Sequence
  CDR2
AIRLSGNRHYAESVKG

SEQ ID NO: 237 - protein, 18 aa, Artificial Sequence
  CDR2
AITWRSGGSAYYADSVKG

SEQ ID NO: 238 - protein, 32 aa, Artificial Sequence
  FR3
RFTISADISKKTMYLQMNSLRPEDTAVYYCLL

SEQ ID NO: 239 - protein, 32 aa, Artificial Sequence
  FR3
RFTISADISKNTMYLQMNSLRPEDTAVYYCLL

SEQ ID NO: 240 - protein, 32 aa, Artificial Sequence
  FR3
RFTISRDNSKNTVYLQMNSLRPEDTAVYYCNA

SEQ ID NO: 241 - protein, 32 aa, Artificial Sequence
  FR3
RFTISRANSKNTVYLQMNSLRPEDTAVYYCKV

SEQ ID NO: 242 - protein, 32 aa, Artificial Sequence
  FR3
RFTISRDNSKNTVYLQMNSLRPEDTAVYYCAA

SEQ ID NO: 243 - protein, 32 aa, Artificial Sequence
  FR3
RFTISRDNSKNTLYLQMNSLRPEDTAVYYCAA

SEQ ID NO: 244 - protein, 32 aa, Artificial Sequence
  FR3
RFTISRDNSKPTMYLQMNSLRPEDTAVYYCHA

SEQ ID NO: 245 - protein, 11 aa, Artificial Sequence
  FR4
WGQGTLVTVSS

SEQ ID NO: 246 - protein, 5 aa, Artificial Sequence
  CDR1
TYWMY

SEQ ID NO: 247 - protein, 14 aa, Artificial Sequence
  FR2
WYRQAPGKQREGVA

SEQ ID NO: 248 - protein, 5 aa, Artificial Sequence
  CDR1
INAMG